European Patent Specification EP 4 056 694 B1, published June 17, 2026. Title: Novel type II citrate synthase variant and a method for producing L-lysine using the same. Applicant: CJ CheilJedang Corporation. The sequence listing filed with the application follows.

SEQUENCE LISTING (10 sequences)

SEQ ID NO: 1 - protein, 437 aa, Artificial Sequence
  (A169V)_type II citrate synthase
MFERDIVATDNNKAVLHYPGGEFEMDIIEASEGNNGVVLGKMLSETGLITFDPGYVSTGSTESKITYIDGDAGILRYRGYDIADLAENATFNEVSYLLINGELPTPDELHKFNDEIRHHTLLDEDFKSQFNVFPRDAHPMATLASSVNILSTYYQDQLNPLDEAQLDKVTVRLMAKVPMLAAYAHRARKGAPYMYPDNSLNARENFLRMMFGYPTEPYEIDPIMVKALDKLLILHADHEQNCSTSTVRMIGSAQANMFVSIAGGINALSGPLHGGANQAVLEMLEDIKSNHGGDATEFMNKVKNKEDGVRLMGFGHRVYKNYDPRAAIVKETAHEILEHLGGDDLLDLAIKLEEIALADDYFISRKLYPNVDFYTGLIYRAMGFPTDFFTVLFAIGRLPGWIAHYREQLGAAGNKINRPRQVYTGNESRKLVPREER

SEQ ID NO: 2 - DNA, 1314 bp, Artificial Sequence
  (A169V)_NCgl0795
atgtttgaaagggatatcgtggctactgataacaacaaggctgtcctgcactaccccggtggcgagttcgaaatggacatcatcgaggcttctgagggtaacaacggtgttgtcctgggcaagatgctgtctgagactggactgatcacttttgacccaggttatgtgagcactggctccaccgagtcgaagatcacctacatcgatggcgatgcgggaatcctgcgttaccgcggctatgacatcgctgatctggctgagaatgccaccttcaacgaggtttcttacctacttatcaacggtgagctaccaaccccagatgagcttcacaagtttaacgacgagattcgccaccacacccttctggacgaggacttcaagtcccagttcaacgtgttcccacgcgacgctcacccaatggcaaccttggcttcctcggttaacattttgtctacctactaccaggaccagctgaacccactcgatgaggcacagcttgataaggtaaccgttcgcctcatggcaaaggttccaatgctggctgcgtacgcacaccgcgcacgcaagggtgctccttacatgtacccagacaactccctcaatgcgcgtgagaacttcctgcgcatgatgttcggttacccaaccgagccatacgagatcgacccaatcatggtcaaggctctggacaagctgctcatcctgcacgctgaccacgagcagaactgctccacctccaccgttcgtatgatcggttccgcacaggccaacatgtttgtctccatcgctggtggcatcaacgctctgtccggcccactgcacggtggcgcaaaccaggctgttctggagatgctcgaagacatcaagagcaaccacggtggcgacgcaaccgagttcatgaacaaggtcaagaacaaggaagacggcgtccgcctcatgggcttcggacaccgcgtttacaagaactacgatccacgtgcagcaatcgtcaaggagaccgcacacgagatcctcgagcacctcggtggcgacgatcttctggatctggcaatcaagctggaagaaattgcactggctgatgattacttcatctcccgcaagctctacccgaacgtagacttctacaccggcctgatctaccgcgcaatgggcttcccaactgacttcttcaccgtattgttcgcaatcggtcgtctgccaggatggatcgctcactaccgcgagcagctcggtgcagcaggcaacaagatcaaccgcccacgccaggtctacaccggcaacgaatcccgcaagttggttcctcgcgaggagcgctaa

SEQ ID NO: 3 - protein, 437 aa, Artificial Sequence [sequence omitted]

SEQ ID NO: 4 - DNA, 1314 bp, Artificial Sequence
  (WT)_NCgl0795
atgtttgaaagggatatcgtggctactgataacaacaaggctgtcctgcactaccccggtggcgagttcgaaatggacatcatcgaggcttctgagggtaacaacggtgttgtcctgggcaagatgctgtctgagactggactgatcacttttgacccaggttatgtgagcactggctccaccgagtcgaagatcacctacatcgatggcgatgcgggaatcctgcgttaccgcggctatgacatcgctgatctggctgagaatgccaccttcaacgaggtttcttacctacttatcaacggtgagctaccaaccccagatgagcttcacaagtttaacgacgagattcgccaccacacccttctggacgaggacttcaagtcccagttcaacgtgttcccacgcgacgctcacccaatggcaaccttggcttcctcggttaacattttgtctacctactaccaggaccagctgaacccactcgatgaggcacagcttgataaggcaaccgttcgcctcatggcaaaggttccaatgctggctgcgtacgcacaccgcgcacgcaagggtgctccttacatgtacccagacaactccctcaatgcgcgtgagaacttcctgcgcatgatgttcggttacccaaccgagccatacgagatcgacccaatcatggtcaaggctctggacaagctgctcatcctgcacgctgaccacgagcagaactgctccacctccaccgttcgtatgatcggttccgcacaggccaacatgtttgtctccatcgctggtggcatcaacgctctgtccggcccactgcacggtggcgcaaaccaggctgttctggagatgctcgaagacatcaagagcaaccacggtggcgacgcaaccgagttcatgaacaaggtcaagaacaaggaagacggcgtccgcctcatgggcttcggacaccgcgtttacaagaactacgatccacgtgcagcaatcgtcaaggagaccgcacacgagatcctcgagcacctcggtggcgacgatcttctggatctggcaatcaagctggaagaaattgcactggctgatgattacttcatctcccgcaagctctacccgaacgtagacttctacaccggcctgatctaccgcgcaatgggcttcccaactgacttcttcaccgtattgttcgcaatcggtcgtctgccaggatggatcgctcactaccgcgagcagctcggtgcagcaggcaacaagatcaaccgcccacgccaggtctacaccggcaacgaatcccgcaagttggttcctcgcgaggagcgctaa

SEQ ID NO: 5 - DNA, 39 bp, Artificial Sequence
  NCgl0795_1F
tgaattcgagctcggtacccaacaaatatgtttgaaagg

SEQ ID NO: 6 - DNA, 33 bp, Artificial Sequence
  NCgl0795_2R
catgaggcgaacggttaccttatcaagctgtgc

SEQ ID NO: 7 - DNA, 33 bp, Artificial Sequence
  NCgl0795_3F
gcacagcttgataaggtaaccgttcgcctcatg

SEQ ID NO: 8 - DNA, 40 bp, Artificial Sequence
  NCgl0795_4R
gtcgactctagaggatccccttcttccagcttgattgcca

SEQ ID NO: 9 - DNA, 19 bp, Artificial Sequence
  NCgl0795_5F
aacaaatatgtttgaaagg

SEQ ID NO: 10 - DNA, 20 bp, Artificial Sequence
  NCgl0795_6R
ttcttccagcttgattgcca